European Patent Application EP 4 686 470 A1, published February 4, 2026. Title: MACROCYCLIC PEPTIDOMIMETICS AS ANTIVIRAL AGENTS. Applicant: Ospedale San Raffaele s.r.l. The sequence listing filed with the application follows.

SEQUENCE LISTING (3 sequences)

SEQ ID NO: 1 - protein, 13 aa, synthetic construct
KTSAVLQSGFRKM

SEQ ID NO: 2 - DNA, 21 bp, synthetic construct
  source 1..21: mol_type = other DNA
gtgtttattttgcttccactg

SEQ ID NO: 3 - DNA, 21 bp, synthetic construct
  source 1..21: mol_type = other DNA
ggctgagagacatattcaaaa